European Patent Specification EP 3 371 212 B1, published October 11, 2023. Title: Peptides and Method for Treatment of Cardiac Arrest. Applicant: THE BOARD OF TRUSTEES OF THE  UNIVERSITY OF ILLINOIS Vanden Hoek, Terry Xhu, Xiangdong Li, Jing. The sequence listing filed with the application follows.

SEQUENCE LISTING (208 sequences)

SEQ ID NO: 1 - protein, 9 aa, Artificial Sequence
  Synthetic peptide
  MISC_FEATURE (4)..(4): Xaa denotes Ser or Thr
BQHXQITKV

SEQ ID NO: 2 - protein, 9 aa, Artificial Sequence
  Synthetic peptide
  MISC_FEATURE (4)..(4): Xaa denotes Cys or Tyr
LPBXYBTPL

SEQ ID NO: 3 - protein, 9 aa, Artificial Sequence
  Synthetic peptide
  MISC_FEATURE (2)..(2): Xaa denotes Arg or His
  MISC_FEATURE (7)..(7): Xaa denotes Ile or Val
FXBFBYXAB

SEQ ID NO: 4 - protein, 9 aa, Artificial Sequence
  Synthetic peptide
DQHSQITKV

SEQ ID NO: 5 - protein, 9 aa, Artificial Sequence
  Synthetic peptide
DQHTQITKV

SEQ ID NO: 6 - protein, 9 aa, Artificial Sequence
  Synthetic peptide
NQHSQITKV

SEQ ID NO: 7 - protein, 9 aa, Artificial Sequence
  Synthetic peptide
NQHTQITKV

SEQ ID NO: 8 - protein, 9 aa, Artificial Sequence
  Synthetic peptide
LPDCYDTPL

SEQ ID NO: 9 - protein, 9 aa, Artificial Sequence
  Synthetic peptide
LPDYYDTPL

SEQ ID NO: 10 - protein, 9 aa, Artificial Sequence
  Synthetic peptide
LPNCYDTPL

SEQ ID NO: 11 - protein, 9 aa, Artificial Sequence
  Synthetic peptide
LPNYYDTPL

SEQ ID NO: 12 - protein, 9 aa, Artificial Sequence
  Synthetic peptide
LPDCYNTPL

SEQ ID NO: 13 - protein, 9 aa, Artificial Sequence
  Synthetic peptide
LPDYYNTPL

SEQ ID NO: 14 - protein, 9 aa, Artificial Sequence
  Synthetic peptide
LPNCYNTPL

SEQ ID NO: 15 - protein, 9 aa, Artificial Sequence
  Synthetic peptide
LPNYYNTPL

SEQ ID NO: 16 - protein, 9 aa, Artificial Sequence
  Synthetic peptide
FHDFDYVAD

SEQ ID NO: 17 - protein, 9 aa, Artificial Sequence
  Synthetic peptide
FRDFDYIAD

SEQ ID NO: 18 - protein, 9 aa, Artificial Sequence
  Synthetic peptide
FHNFDYVAD

SEQ ID NO: 19 - protein, 9 aa, Artificial Sequence
  Synthetic peptide
FRNFDYIAD

SEQ ID NO: 20 - protein, 9 aa, Artificial Sequence
  Synthetic peptide
FHDFNYVAD

SEQ ID NO: 21 - protein, 9 aa, Artificial Sequence
  Synthetic peptide
FRDFNYIAD

SEQ ID NO: 22 - protein, 9 aa, Artificial Sequence
  Synthetic peptide
FHDFDYVAN

SEQ ID NO: 23 - protein, 9 aa, Artificial Sequence
  Synthetic peptide
FRDFDYIAN

SEQ ID NO: 24 - protein, 9 aa, Artificial Sequence
  Synthetic peptide
FHNFNYVAD

SEQ ID NO: 25 - protein, 9 aa, Artificial Sequence
  Synthetic peptide
FRNFNYIAD

SEQ ID NO: 26 - protein, 9 aa, Artificial Sequence
  Synthetic peptide
FHNFDYVAN

SEQ ID NO: 27 - protein, 9 aa, Artificial Sequence
  Synthetic peptide
FRNFDYIAN

SEQ ID NO: 28 - protein, 9 aa, Artificial Sequence
  Synthetic peptide
FHDFNYVAN

SEQ ID NO: 29 - protein, 9 aa, Artificial Sequence
  Synthetic peptide
FRDFNYIAN

SEQ ID NO: 30 - protein, 15 aa, Artificial Sequence
  Synthetic peptide
NEPFDEDQHTQITKV

SEQ ID NO: 31 - protein, 18 aa, Artificial Sequence
  Synthetic peptide
KLALKLALKALKAALKLA

SEQ ID NO: 32 - protein, 16 aa, Artificial Sequence
  Synthetic peptide
  MISC_FEATURE (1)..(1): Xaa is present or absent and when present denotes Lys or Val
  MISC_FEATURE (2)..(2): Xaa is present or absent and when present denotes Lys
  MISC_FEATURE (8)..(8): Xaa denotes any amino acid residue
  MISC_FEATURE (11)..(11): Xaa is present or absent and when present denotes Lys
  MISC_FEATURE (12)..(12): Xaa is present or absent and when present denotes Ile
  MISC_FEATURE (13)..(16): Xaa is present or absent and when present denotes any amino acid residue
XXKKKIKXEIXXXXXX

SEQ ID NO: 33 - protein, 12 aa, Artificial Sequence
  Synthetic peptide
VKKKKIKREIKI

SEQ ID NO: 34 - protein, 12 aa, Artificial Sequence
  Synthetic peptide
VKKKKIKNEIKI

SEQ ID NO: 35 - protein, 12 aa, Artificial Sequence
  Synthetic peptide
VKKKKIKAEIKI

SEQ ID NO: 36 - protein, 12 aa, Artificial Sequence
  Synthetic peptide
VKKKKIKKEIKI

SEQ ID NO: 37 - protein, 18 aa, Artificial Sequence
  Synthetic peptide
RQKRLIRQKRLIRQKRLI

SEQ ID NO: 38 - protein, 18 aa, Artificial Sequence
  Synthetic peptide
RHSRIGRHSRIGRHSRIG

SEQ ID NO: 39 - protein, 16 aa, Artificial Sequence
  Synthetic peptide
RHSRIGIIQQRRTRNG

SEQ ID NO: 40 - protein, 16 aa, Artificial Sequence
  Synthetic peptide
RHSRIGVTRQRRARNG

SEQ ID NO: 41 - protein, 15 aa, Artificial Sequence
  Synthetic peptide
RRRRRRRSRGRRRTY

SEQ ID NO: 42 - protein, 9 aa, Artificial Sequence
  Synthetic peptide
RKKRRQRRR

SEQ ID NO: 43 - protein, 11 aa, Artificial Sequence
  Synthetic peptide
YGRKKRRQRRR

SEQ ID NO: 44 - protein, 9 aa, Artificial Sequence
  Synthetic peptide
RRRRRRRRR

SEQ ID NO: 45 - protein, 11 aa, Artificial Sequence
  Synthetic peptide
RRRRRRRRRRR

SEQ ID NO: 46 - protein, 32 aa, Artificial Sequence
  Synthetic peptide
GLFEAIEGFIENGWEGMIDGWYGRRRRRRRRR

SEQ ID NO: 47 - protein, 16 aa, Artificial Sequence
  Synthetic peptide
RQIKIWFQNRRMKWKK

SEQ ID NO: 48 - protein, 27 aa, Artificial Sequence
  Synthetic peptide
GWTLNSAGYLLGKINLKALAALAKKIL

SEQ ID NO: 49 - protein, 33 aa, Artificial Sequence
  Synthetic peptide
GDCLPHLKLCKENKDCCSKKCKRRGTNIEKRCR

SEQ ID NO: 50 - protein, 10 aa, Artificial Sequence
  Synthetic peptide
KKKKKKKKKK

SEQ ID NO: 51 - protein, 9 aa, Artificial Sequence
  Synthetic peptide
KKKKKKKKK

SEQ ID NO: 52 - protein, 11 aa, Artificial Sequence
  Synthetic peptide
YARAAARQARA

SEQ ID NO: 53 - protein, 12 aa, Artificial Sequence
  Synthetic peptide
PLSSIFSRIGDP

SEQ ID NO: 54 - protein, 27 aa, Artificial Sequence
  Synthetic peptide
MANLGYWLLALFVMWTDVGLCKKRPKP

SEQ ID NO: 55 - protein, 35 aa, Artificial Sequence
  Synthetic peptide
GGGARKKAAKAARKKAAKAARKKAAKAARKKAAKA

SEQ ID NO: 56 - protein, 19 aa, Artificial Sequence
  Synthetic peptide
LLIILRRRRIRKQAHAHSK

SEQ ID NO: 57 - protein, 23 aa, Artificial Sequence
  Synthetic peptide
LIRLWSHLIHIWFQNRRLKWKKK

SEQ ID NO: 58 - protein, 22 aa, Artificial Sequence
  Synthetic peptide
TPWWRLWTKWHHKRRDLPRKPE

SEQ ID NO: 59 - protein, 20 aa, Artificial Sequence
  Synthetic peptide
GLWRALWRLLRSLWRLLWRA

SEQ ID NO: 60 - protein, 23 aa, Artificial Sequence
  Synthetic peptide
DSHAKRHHGYRKFHEKHHSHRGY

SEQ ID NO: 61 - protein, 16 aa, Artificial Sequence
  Synthetic peptide
KKKEERADLIAYLKKA

SEQ ID NO: 62 - protein, 16 aa, Artificial Sequence
  Synthetic peptide
GLRKRLRKFRNKIKEK

SEQ ID NO: 63 - protein, 20 aa, Artificial Sequence
  Synthetic peptide
YGRKKRRQRRRLPDCYDTPL

SEQ ID NO: 64 - protein, 18 aa, Artificial Sequence
  Synthetic peptide
RRRRRRRRRLPDCYDTPL

SEQ ID NO: 65 - protein, 18 aa, Artificial Sequence
  Synthetic peptide
KKKKKKKKKLPDCYDTPL

SEQ ID NO: 66 - protein, 20 aa, Artificial Sequence
  Synthetic peptide
  MOD_RES (20)..(20): AMIDATION
YGRKKRRQRRRLPDCYDTPL

SEQ ID NO: 67 - protein, 18 aa, Artificial Sequence
  Synthetic peptide
  MOD_RES (18)..(18): AMIDATION
RRRRRRRRRLPDCYDTPL

SEQ ID NO: 68 - protein, 18 aa, Artificial Sequence
  Synthetic peptide
  MOD_RES (18)..(18): AMIDATION
KKKKKKKKKLPDCYDTPL

SEQ ID NO: 69 - protein, 9 aa, Artificial Sequence
  Synthetic peptide
  MOD_RES (1)..(1): Myristoylation
LPDCYDTPL

SEQ ID NO: 70 - protein, 9 aa, Artificial Sequence
  Synthetic peptide
  MOD_RES (9)..(9): AMIDATION
LPDCYDTPL

SEQ ID NO: 71 - protein, 9 aa, Artificial Sequence
  Synthetic peptide
  MOD_RES (1)..(1): Myristoylation
  MOD_RES (9)..(9): AMIDATION
LPDCYDTPL

SEQ ID NO: 72 - protein, 10 aa, Artificial Sequence
  Synthetic peptide
  MOD_RES (1)..(1): Myristoylation
GLPDCYDTPL

SEQ ID NO: 73 - protein, 10 aa, Artificial Sequence
  Synthetic peptide
  MOD_RES (10)..(10): AMIDATION
GLPDCYDTPL

SEQ ID NO: 74 - protein, 10 aa, Artificial Sequence
  Synthetic peptide
  MOD_RES (1)..(1): Myristoylation
  MOD_RES (10)..(10): AMIDATION
GLPDCYDTPL

SEQ ID NO: 75 - protein, 20 aa, Artificial Sequence
  Synthetic peptide
YGRKKRRQRRRLPNCYNTPL

SEQ ID NO: 76 - protein, 18 aa, Artificial Sequence
  Synthetic peptide
RRRRRRRRRLPNCYNTPL

SEQ ID NO: 77 - protein, 18 aa, Artificial Sequence
  Synthetic peptide
KKKKKKKKKLPNCYNTPL

SEQ ID NO: 78 - protein, 20 aa, Artificial Sequence
  Synthetic peptide
  MOD_RES (20)..(20): AMIDATION
YGRKKRRQRRRLPNCYNTPL

SEQ ID NO: 79 - protein, 18 aa, Artificial Sequence
  Synthetic peptide
  MOD_RES (18)..(18): AMIDATION
RRRRRRRRRLPNCYNTPL

SEQ ID NO: 80 - protein, 18 aa, Artificial Sequence
  Synthetic peptide
  MOD_RES (18)..(18): AMIDATION
KKKKKKKKKLPNCYNTPL

SEQ ID NO: 81 - protein, 9 aa, Artificial Sequence
  Synthetic peptide
  MOD_RES (9)..(9): AMIDATION
LPNCYNTPL

SEQ ID NO: 82 - protein, 9 aa, Artificial Sequence
  Synthetic peptide
  MOD_RES (1)..(1): Myristoylation
  MOD_RES (9)..(9): AMIDATION
LPNCYNTPL

SEQ ID NO: 83 - protein, 9 aa, Artificial Sequence
  Synthetic peptide
  MOD_RES (1)..(1): Myristoylation
LPNCYNTPL

SEQ ID NO: 84 - protein, 10 aa, Artificial Sequence
  Synthetic peptide
  MOD_RES (10)..(10): AMIDATION
GLPNCYNTPL

SEQ ID NO: 85 - protein, 10 aa, Artificial Sequence
  Synthetic peptide
  MOD_RES (1)..(1): Myristoylation
  MOD_RES (10)..(10): AMIDATION
GLPNCYNTPL

SEQ ID NO: 86 - protein, 10 aa, Artificial Sequence
  Synthetic peptide
  MOD_RES (1)..(1): Myristoylation
GLPNCYNTPL

SEQ ID NO: 87 - protein, 20 aa, Artificial Sequence
  Synthetic peptide
YGRKKRRQRRRLPDYYDTPL

SEQ ID NO: 88 - protein, 18 aa, Artificial Sequence
  Synthetic peptide
RRRRRRRRRLPDYYDTPL

SEQ ID NO: 89 - protein, 18 aa, Artificial Sequence
  Synthetic peptide
KKKKKKKKKLPDYYDTPL

SEQ ID NO: 90 - protein, 20 aa, Artificial Sequence
  Synthetic peptide
  MOD_RES (20)..(20): AMIDATION
YGRKKRRQRRRLPDYYDTPL

SEQ ID NO: 91 - protein, 18 aa, Artificial Sequence
  Synthetic peptide
  MOD_RES (18)..(18): AMIDATION
RRRRRRRRRLPDYYDTPL

SEQ ID NO: 92 - protein, 18 aa, Artificial Sequence
  Synthetic peptide
  MOD_RES (18)..(18): AMIDATION
KKKKKKKKKLPDYYDTPL

SEQ ID NO: 93 - protein, 9 aa, Artificial Sequence
  Synthetic peptide
  MOD_RES (9)..(9): AMIDATION
LPDYYDTPL

SEQ ID NO: 94 - protein, 9 aa, Artificial Sequence
  Synthetic peptide
  MOD_RES (1)..(1): Myristoylation
  MOD_RES (9)..(9): AMIDATION
LPDYYDTPL

SEQ ID NO: 95 - protein, 9 aa, Artificial Sequence
  Synthetic peptide
  MOD_RES (1)..(1): Myristoylation
LPDYYDTPL

SEQ ID NO: 96 - protein, 10 aa, Artificial Sequence
  Synthetic peptide
  MOD_RES (10)..(10): AMIDATION
GLPDYYDTPL

SEQ ID NO: 97 - protein, 10 aa, Artificial Sequence
  Synthetic peptide
  MOD_RES (1)..(1): Myristoylation
  MOD_RES (10)..(10): AMIDATION
GLPDYYDTPL

SEQ ID NO: 98 - protein, 10 aa, Artificial Sequence
  Synthetic peptide
  MOD_RES (1)..(1): Myristoylation
GLPDYYDTPL

SEQ ID NO: 99 - protein, 20 aa, Artificial Sequence
  Synthetic peptide
YGRKKRRQRRRLPNYYNTPL

SEQ ID NO: 100 - protein, 18 aa, Artificial Sequence
  Synthetic peptide
RRRRRRRRRLPNYYNTPL

SEQ ID NO: 101 - protein, 18 aa, Artificial Sequence
  Synthetic peptide
KKKKKKKKKLPNYYNTPL

SEQ ID NO: 102 - protein, 20 aa, Artificial Sequence
  Synthetic peptide
  MOD_RES (20)..(20): AMIDATION
YGRKKRRQRRRLPNYYNTPL

SEQ ID NO: 103 - protein, 18 aa, Artificial Sequence
  Synthetic peptide
  MOD_RES (18)..(18): AMIDATION
RRRRRRRRRLPNYYNTPL

SEQ ID NO: 104 - protein, 18 aa, Artificial Sequence
  Synthetic peptide
  MOD_RES (18)..(18): AMIDATION
KKKKKKKKKLPNYYNTPL

SEQ ID NO: 105 - protein, 9 aa, Artificial Sequence
  Synthetic peptide
  MOD_RES (9)..(9): AMIDATION
LPNYYNTPL

SEQ ID NO: 106 - protein, 9 aa, Artificial Sequence
  Synthetic peptide
  MOD_RES (1)..(1): Myristoylation
  MOD_RES (9)..(9): AMIDATION
LPNYYNTPL

SEQ ID NO: 107 - protein, 9 aa, Artificial Sequence
  Synthetic peptide
  MOD_RES (1)..(1): Myristoylation
LPNYYNTPL

SEQ ID NO: 108 - protein, 10 aa, Artificial Sequence
  Synthetic peptide
  MOD_RES (10)..(10): AMIDATION
GLPNYYNTPL

SEQ ID NO: 109 - protein, 10 aa, Artificial Sequence
  Synthetic peptide
  MOD_RES (1)..(1): Myristoylation
  MOD_RES (10)..(10): AMIDATION
GLPNYYNTPL

SEQ ID NO: 110 - protein, 10 aa, Artificial Sequence
  Synthetic peptide
  MOD_RES (1)..(1): Myristoylation
GLPNYYNTPL

SEQ ID NO: 111 - protein, 20 aa, Artificial Sequence
  Synthetic peptide
YGRKKRRQRRRDQHSQITKV

SEQ ID NO: 112 - protein, 18 aa, Artificial Sequence
  Synthetic peptide
RRRRRRRRRDQHSQITKV

SEQ ID NO: 113 - protein, 18 aa, Artificial Sequence
  Synthetic peptide
KKKKKKKKKDQHSQITKV

SEQ ID NO: 114 - protein, 20 aa, Artificial Sequence
  Synthetic peptide
  MOD_RES (20)..(20): AMIDATION
YGRKKRRQRRRDQHSQITKV

SEQ ID NO: 115 - protein, 18 aa, Artificial Sequence
  Synthetic peptide
  MOD_RES (18)..(18): AMIDATION
RRRRRRRRRDQHSQITKV

SEQ ID NO: 116 - protein, 18 aa, Artificial Sequence
  Synthetic peptide
  MOD_RES (18)..(18): AMIDATION
KKKKKKKKKDQHSQITKV

SEQ ID NO: 117 - protein, 9 aa, Artificial Sequence
  Synthetic peptide
  MOD_RES (9)..(9): AMIDATION
DQHSQITKV

SEQ ID NO: 118 - protein, 9 aa, Artificial Sequence
  Synthetic peptide
  MOD_RES (1)..(1): Myristoylation
  MOD_RES (9)..(9): AMIDATION
DQHSQITKV

SEQ ID NO: 119 - protein, 9 aa, Artificial Sequence
  Synthetic peptide
  MOD_RES (1)..(1): Myristoylation
DQHSQITKV

SEQ ID NO: 120 - protein, 10 aa, Artificial Sequence
  Synthetic peptide
  MOD_RES (10)..(10): AMIDATION
GDQHSQITKV

SEQ ID NO: 121 - protein, 10 aa, Artificial Sequence
  Synthetic peptide
  MOD_RES (1)..(1): Myristoylation
  MOD_RES (10)..(10): AMIDATION
GDQHSQITKV

SEQ ID NO: 122 - protein, 10 aa, Artificial Sequence
  Synthetic peptide
  MOD_RES (1)..(1): Myristoylation
GDQHSQITKV

SEQ ID NO: 123 - protein, 20 aa, Artificial Sequence
  Synthetic peptide
YGRKKRRQRRRNQHSQITKV

SEQ ID NO: 124 - protein, 18 aa, Artificial Sequence
  Synthetic peptide
RRRRRRRRRNQHSQITKV

SEQ ID NO: 125 - protein, 18 aa, Artificial Sequence
  Synthetic peptide
KKKKKKKKKNQHSQITKV

SEQ ID NO: 126 - protein, 20 aa, Artificial Sequence
  Synthetic peptide
  MOD_RES (20)..(20): AMIDATION
YGRKKRRQRRRNQHSQITKV

SEQ ID NO: 127 - protein, 18 aa, Artificial Sequence
  Synthetic peptide
  MOD_RES (18)..(18): AMIDATION
RRRRRRRRRNQHSQITKV

SEQ ID NO: 128 - protein, 18 aa, Artificial Sequence
  Synthetic peptide
  MOD_RES (18)..(18): AMIDATION
KKKKKKKKKNQHSQITKV

SEQ ID NO: 129 - protein, 9 aa, Artificial Sequence
  Synthetic peptide
  MOD_RES (9)..(9): AMIDATION
NQHSQITKV

SEQ ID NO: 130 - protein, 9 aa, Artificial Sequence
  Synthetic peptide
  MOD_RES (1)..(1): Myristoylation
  MOD_RES (9)..(9): AMIDATION
NQHSQITKV

SEQ ID NO: 131 - protein, 9 aa, Artificial Sequence
  Synthetic peptide
  MOD_RES (1)..(1): Myristoylation
NQHSQITKV

SEQ ID NO: 132 - protein, 10 aa, Artificial Sequence
  Synthetic peptide
  MOD_RES (10)..(10): AMIDATION
GNQHSQITKV

SEQ ID NO: 133 - protein, 10 aa, Artificial Sequence
  Synthetic peptide
  MOD_RES (1)..(1): Myristoylation
  MOD_RES (10)..(10): AMIDATION
GNQHSQITKV

SEQ ID NO: 134 - protein, 10 aa, Artificial Sequence
  Synthetic peptide
  MOD_RES (1)..(1): Myristoylation
GNQHSQITKV

SEQ ID NO: 135 - protein, 20 aa, Artificial Sequence
  Synthetic peptide
YGRKKRRQRRRDQHTQITKV

SEQ ID NO: 136 - protein, 18 aa, Artificial Sequence
  Synthetic peptide
RRRRRRRRRDQHTQITKV

SEQ ID NO: 137 - protein, 18 aa, Artificial Sequence
  Synthetic peptide
KKKKKKKKKDQHTQITKV

SEQ ID NO: 138 - protein, 20 aa, Artificial Sequence
  Synthetic peptide
  MOD_RES (20)..(20): AMIDATION
YGRKKRRQRRRDQHTQITKV

SEQ ID NO: 139 - protein, 18 aa, Artificial Sequence
  Synthetic peptide
  MOD_RES (18)..(18): AMIDATION
RRRRRRRRRDQHTQITKV

SEQ ID NO: 140 - protein, 18 aa, Artificial Sequence
  Synthetic peptide
  MOD_RES (18)..(18): AMIDATION
KKKKKKKKKDQHTQITKV

SEQ ID NO: 141 - protein, 9 aa, Artificial Sequence
  Synthetic peptide
  MOD_RES (9)..(9): AMIDATION
DQHTQITKV

SEQ ID NO: 142 - protein, 10 aa, Artificial Sequence
  Synthetic peptide
  MOD_RES (1)..(1): Myristoylation
  MOD_RES (10)..(10): AMIDATION
DQHTQITKVV

SEQ ID NO: 143 - protein, 9 aa, Artificial Sequence
  Synthetic peptide
  MOD_RES (1)..(1): Myristoylation
DQHTQITKV

SEQ ID NO: 144 - protein, 10 aa, Artificial Sequence
  Synthetic peptide
  MOD_RES (10)..(10): AMIDATION
GDQHTQITKV

SEQ ID NO: 145 - protein, 10 aa, Artificial Sequence
  Synthetic peptide
  MOD_RES (1)..(1): Myristoylation
  MOD_RES (10)..(10): AMIDATION
GDQHTQITKV

SEQ ID NO: 146 - protein, 10 aa, Artificial Sequence
  Synthetic peptide
  MOD_RES (1)..(1): Myristoylation
GDQHTQITKV

SEQ ID NO: 147 - protein, 20 aa, Artificial Sequence
  Synthetic peptide
YGRKKRRQRRRNQHTQITKV

SEQ ID NO: 148 - protein, 18 aa, Artificial Sequence
  Synthetic peptide
RRRRRRRRRNQHTQITKV

SEQ ID NO: 149 - protein, 18 aa, Artificial Sequence
  Synthetic peptide
KKKKKKKKKNQHTQITKV

SEQ ID NO: 150 - protein, 20 aa, Artificial Sequence
  Synthetic peptide
  MOD_RES (20)..(20): AMIDATION
YGRKKRRQRRRNQHTQITKV

SEQ ID NO: 151 - protein, 18 aa, Artificial Sequence
  Synthetic peptide
  MOD_RES (18)..(18): AMIDATION
RRRRRRRRRNQHTQITKV

SEQ ID NO: 152 - protein, 18 aa, Artificial Sequence
  Synthetic peptide
  MOD_RES (18)..(18): AMIDATION
KKKKKKKKKNQHTQITKV

SEQ ID NO: 153 - protein, 9 aa, Artificial Sequence
  Synthetic peptide
  MOD_RES (9)..(9): AMIDATION
NQHTQITKV

SEQ ID NO: 154 - protein, 9 aa, Artificial Sequence
  Synthetic peptide
  MOD_RES (1)..(1): Myristoylation
  MOD_RES (9)..(9): AMIDATION
NQHTQITKV

SEQ ID NO: 155 - protein, 9 aa, Artificial Sequence
  Synthetic peptide
  MOD_RES (1)..(1): Myristoylation
NQHTQITKV

SEQ ID NO: 156 - protein, 10 aa, Artificial Sequence
  Synthetic peptide
  MOD_RES (10)..(10): AMIDATION
GNQHTQITKV

SEQ ID NO: 157 - protein, 10 aa, Artificial Sequence
  Synthetic peptide
  MOD_RES (1)..(1): Myristoylation
  MOD_RES (10)..(10): AMIDATION
GNQHTQITKV

SEQ ID NO: 158 - protein, 10 aa, Artificial Sequence
  Synthetic peptide
  MOD_RES (1)..(1): Myristoylation
GNQHSQITKV

SEQ ID NO: 159 - protein, 20 aa, Artificial Sequence
  Synthetic peptide
YGRKKRRQRRRFHDFDYVAD

SEQ ID NO: 160 - protein, 18 aa, Artificial Sequence
  Synthetic peptide
RRRRRRRRRFHDFDYVAD

SEQ ID NO: 161 - protein, 18 aa, Artificial Sequence
  Synthetic peptide
KKKKKKKKKFHDFDYVAD

SEQ ID NO: 162 - protein, 20 aa, Artificial Sequence
  Synthetic peptide
  MOD_RES (20)..(20): AMIDATION
YGRKKRRQRRRFHDFDYVAD

SEQ ID NO: 163 - protein, 18 aa, Artificial Sequence
  Synthetic peptide
  MOD_RES (18)..(18): AMIDATION
RRRRRRRRRFHDFDYVAD

SEQ ID NO: 164 - protein, 18 aa, Artificial Sequence
  Synthetic peptide
  MOD_RES (18)..(18): AMIDATION
KKKKKKKKKFHDFDYVAD

SEQ ID NO: 165 - protein, 9 aa, Artificial Sequence
  Synthetic peptide
  MOD_RES (9)..(9): AMIDATION
FHDFDYVAD

SEQ ID NO: 166 - protein, 9 aa, Artificial Sequence
  Synthetic peptide
  MOD_RES (1)..(1): Myristoylation
  MOD_RES (9)..(9): AMIDATION
FHDFDYVAD

SEQ ID NO: 167 - protein, 9 aa, Artificial Sequence
  Synthetic peptide
  MOD_RES (1)..(1): Myristoylation
FHDFDYVAD

SEQ ID NO: 168 - protein, 10 aa, Artificial Sequence
  Synthetic peptide
  MOD_RES (10)..(10): AMIDATION
GFHDFDYVAD

SEQ ID NO: 169 - protein, 10 aa, Artificial Sequence
  Synthetic peptide
  MOD_RES (1)..(1): Myristoylation
  MOD_RES (10)..(10): AMIDATION
GFHDFDYVAD

SEQ ID NO: 170 - protein, 10 aa, Artificial Sequence
  Synthetic peptide
  MOD_RES (1)..(1): Myristoylation
GFHDFDYVAD

SEQ ID NO: 171 - protein, 20 aa, Artificial Sequence
  Synthetic peptide
YGRKKRRQRRRFHNFNYVAN

SEQ ID NO: 172 - protein, 18 aa, Artificial Sequence
  Synthetic peptide
RRRRRRRRRFHNFNYVAN

SEQ ID NO: 173 - protein, 18 aa, Artificial Sequence
  Synthetic peptide
KKKKKKKKKFHNFNYVAN

SEQ ID NO: 174 - protein, 20 aa, Artificial Sequence
  Synthetic peptide
  MOD_RES (20)..(20): AMIDATION
YGRKKRRQRRRFHNFNYVAN

SEQ ID NO: 175 - protein, 18 aa, Artificial Sequence
  Synthetic peptide
  MOD_RES (18)..(18): AMIDATION
RRRRRRRRRFHNFNYVAN

SEQ ID NO: 176 - protein, 18 aa, Artificial Sequence
  Synthetic peptide
  MOD_RES (18)..(18): AMIDATION
KKKKKKKKKFHNFNYVAN

SEQ ID NO: 177 - protein, 9 aa, Artificial Sequence
  Synthetic peptide
  MOD_RES (9)..(9): AMIDATION
FHNFNYVAN

SEQ ID NO: 178 - protein, 9 aa, Artificial Sequence
  Synthetic peptide
  MOD_RES (1)..(1): Myristoylation
  MOD_RES (9)..(9): AMIDATION
FHNFNYVAN

SEQ ID NO: 179 - protein, 9 aa, Artificial Sequence
  Synthetic peptide
  MOD_RES (1)..(1): Myristoylation
FHNFNYVAN

SEQ ID NO: 180 - protein, 10 aa, Artificial Sequence
  Synthetic peptide
  MOD_RES (10)..(10): AMIDATION
GFHNFNYVAN

SEQ ID NO: 181 - protein, 10 aa, Artificial Sequence
  Synthetic peptide
  MOD_RES (1)..(1): Myristoylation
  MOD_RES (10)..(10): AMIDATION
GFHNFNYVAN

SEQ ID NO: 182 - protein, 10 aa, Artificial Sequence
  Synthetic peptide
  MOD_RES (1)..(1): Myristoylation
GFHNFNYVAN

SEQ ID NO: 183 - protein, 20 aa, Artificial Sequence
  Synthetic peptide
YGRKKRRQRRRFRDFDYIAD

SEQ ID NO: 184 - protein, 18 aa, Artificial Sequence
  Synthetic peptide
RRRRRRRRRFRDFDYIAD

SEQ ID NO: 185 - protein, 18 aa, Artificial Sequence
  Synthetic peptide
KKKKKKKKKFRDFDYIAD

SEQ ID NO: 186 - protein, 20 aa, Artificial Sequence
  Synthetic peptide
  MOD_RES (20)..(20): AMIDATION
YGRKKRRQRRRFRDFDYIAD

SEQ ID NO: 187 - protein, 18 aa, Artificial Sequence
  Synthetic peptide
  MOD_RES (18)..(18): AMIDATION
RRRRRRRRRFRDFDYIAD

SEQ ID NO: 188 - protein, 18 aa, Artificial Sequence
  Synthetic peptide
  MOD_RES (18)..(18): AMIDATION
KKKKKKKKKFRDFDYIAD

SEQ ID NO: 189 - protein, 9 aa, Artificial Sequence
  Synthetic peptide
  MOD_RES (9)..(9): AMIDATION
FRDFDYIAD

SEQ ID NO: 190 - protein, 9 aa, Artificial Sequence
  Synthetic peptide
  MOD_RES (1)..(1): Myristoylation
  MOD_RES (9)..(9): AMIDATION
FRDFDYIAD

SEQ ID NO: 191 - protein, 9 aa, Artificial Sequence
  Synthetic peptide
  MOD_RES (1)..(1): Myristoylation
FRDFDYIAD

SEQ ID NO: 192 - protein, 10 aa, Artificial Sequence
  Synthetic peptide
  MOD_RES (10)..(10): AMIDATION
GFRDFDYIAD

SEQ ID NO: 193 - protein, 10 aa, Artificial Sequence
  Synthetic peptide
  MOD_RES (1)..(1): Myristoylation
  MOD_RES (10)..(10): AMIDATION
GFRDFDYIAD

SEQ ID NO: 194 - protein, 10 aa, Artificial Sequence
  Synthetic peptide
  MOD_RES (1)..(1): Myristoylation
GFRDFDYIAD

SEQ ID NO: 195 - protein, 20 aa, Artificial Sequence
  Synthetic peptide
YGRKKRRQRRRFRNFNYIAN

SEQ ID NO: 196 - protein, 18 aa, Artificial Sequence
  Synthetic peptide
RRRRRRRRRFRNFNYIAN

SEQ ID NO: 197 - protein, 18 aa, Artificial Sequence
  Synthetic peptide
KKKKKKKKKFRNFNYIAN

SEQ ID NO: 198 - protein, 20 aa, Artificial Sequence
  Synthetic peptide
  MOD_RES (20)..(20): AMIDATION
YGRKKRRQRRRFRNFNYIAN

SEQ ID NO: 199 - protein, 18 aa, Artificial Sequence
  Synthetic peptide
  MOD_RES (18)..(18): AMIDATION
RRRRRRRRRFRNFNYIAN

SEQ ID NO: 200 - protein, 18 aa, Artificial Sequence
  Synthetic peptide
  MOD_RES (18)..(18): AMIDATION
KKKKKKKKKFRNFNYIAN

SEQ ID NO: 201 - protein, 9 aa, Artificial Sequence
  Synthetic peptide
  MOD_RES (9)..(9): AMIDATION
FRNFNYIAN

SEQ ID NO: 202 - protein, 9 aa, Artificial Sequence
  Synthetic peptide
  MOD_RES (1)..(1): Myristoylation
  MOD_RES (9)..(9): AMIDATION
FRNFNYIAN

SEQ ID NO: 203 - protein, 9 aa, Artificial Sequence
  Synthetic peptide
  MOD_RES (1)..(1): Myristoylation
FRNFNYIAN

SEQ ID NO: 204 - protein, 10 aa, Artificial Sequence
  Synthetic peptide
  MOD_RES (10)..(10): AMIDATION
GFRNFNYIAN

SEQ ID NO: 205 - protein, 10 aa, Artificial Sequence
  Synthetic peptide
  MOD_RES (1)..(1): Myristoylation
  MOD_RES (10)..(10): AMIDATION
GFRNFNYIAN

SEQ ID NO: 206 - protein, 10 aa, Artificial Sequence
  Synthetic peptide
  MOD_RES (1)..(1): Myristoylation
GFRNFNYIAN

SEQ ID NO: 207 - protein, 6 aa, Artificial Sequence
  Synthetic peptide
  MISC_FEATURE (2)..(3): Xaa denotes any amino acid residue.
FXXFDY

SEQ ID NO: 208 - protein, 24 aa, Artificial Sequence
  Synthetic peptide
REPRILSEEEQEMFRDFDYIADWC